European Patent Specification EP 4 023 752 B1, published October 22, 2025. Title: NOVEL PROTEASES AND USES THEREOF. Applicant: CARBIOS. The sequence listing filed with the application follows.

SEQUENCE LISTING (5 sequences)

SEQ ID NO: 1 - protein, 276 aa, ARTIFICIAL SEQUENCE [sequence omitted]

SEQ ID NO: 2 - protein, 81 aa, ARTIFICIAL SEQUENCE
  PROPEPTIDE
APAVPVAMAAAGQGVAGQYIVTLKKGVSVDSTVAKRGIRTQHRFGKVLNGFSAKLTDDQLSKLRTTPGVASIEQDAVITVD

SEQ ID NO: 3 - DNA, 1071 bp, ARTIFICIAL SEQUENCE
  NON MATURED PARENT PROTEIN
gcccccgctgtccccgtcgccatggccgctgccggccagggtgtcgccggccagtacatcgttactctgaagaagggcgtgtctgttgactctaccgttgctaagcgaggcatccgaacccagcaccgattcggaaaggtcctgaacggattttccgccaagctcaccgacgatcagctgtctaagctccgaaccactcccggcgtcgcctctatcgagcaggacgctgttattaccgtcgatgccactcagaacaaccctccctcctggggtctcgaccgaatcgaccagaccaacctgcctctctctcgatcgtacacctacaactctactggagccggcgtcaacgcttacatcattgacaccggaatttacactgcccactccgatttcggcggtcgagctaccaacgtgtacgacgccctgggaggcaacggtcaggattgcaacggtcacggaacccatgtggccggcactgttggtggagccgcttacggtgtcgccaaggctgtgaacctgcgaggtgtccgagtgctcaactgtttcggcctgggtaccctgtccggagtcatcgctggcatgaactgggtggcctctaaccatgttaagcccgccgtcgctaacatgtccctgggcggtggatactcctcttcgctgaacaccgccgctaacaacctcgcttcctctggagtgttcctggccgttgccgctggcaacgagaccactaacgcctgcaaccgatcgcctgcttccgccgctaacgctaccactgtggccgcttcgacctctactgacgcccgagcttcttactcgaactacggttcttgtgttcacctctacgctcccggatcgtccatcacctctgcctggctgaacggcggtaccaacactatttctggcacctcgatggccactcctcatgttgctggtaccgccgctctctacaaggccacttacggagacgcttccttttctaccattcgatcctggctggtgtctaacgccacctcgggtgtcatcactggtaacgtctctggaactcccaacctgctcctgaacaagcgaagcctg

SEQ ID NO: 4 - protein, 22 aa, ARTIFICIAL SEQUENCE
  SIGNAL PEPTIDE
MKYLLPTAAAGLLLLAAQPAMA

SEQ ID NO: 5 - protein, 8 aa, ARTIFICIAL SEQUENCE
  HIS TAG
LEHHHHHH